European Patent Application EP 4 650 450 A1, published November 19, 2025. Title: 抗ネコＰＤ－１抗体. Applicant: 国立大学法人山口大学. The sequence listing filed with the application follows.

SEQUENCE LISTING (23 sequences)

SEQ ID NO: 1 - protein, 5 aa, synthetic construct
  REGION 1..5: note = H Chain CDR1 of 1A1-2 antibody
  REGION 1..5: note = MISC_FEATURE - Inventor: Mizuno Takuya; Nishibori Shoma
DYSIH

SEQ ID NO: 2 - protein, 17 aa, synthetic construct
  REGION 1..17: note = H Chain CDR2 of 1A1-2 antibody
WINTETGEPTYADDFKG

SEQ ID NO: 3 - protein, 15 aa, synthetic construct
  REGION 1..15: note = H Chain CDR3 of 1A1-2 antibody
PLFYYYITSPRSMDC

SEQ ID NO: 4 - protein, 11 aa, synthetic construct
  REGION 1..11: note = L Chain CDR1 of 1A1-2 antibody
KASQSVTNDVA

SEQ ID NO: 5 - protein, 7 aa, synthetic construct
  REGION 1..7: note = L Chain CDR2 of 1A1-2 antibody
YASNRYT

SEQ ID NO: 6 - protein, 9 aa, synthetic construct
  REGION 1..9: note = L Chain CDR3 of 1A1-2 antibody
QQDYSSPYT

SEQ ID NO: 7 - protein, 124 aa, synthetic construct
  REGION 1..124: note = H Chain V Region of 1A1-2 antibody
QIQLVQSGPELKKPGETVKISCKASGYTFTDYSIHWVKQAPGKGLKWMGWINTETGEPTYADDFKGRFAFSLETSVSAAFLQINNLKNEDTATYFCARPLFYYYITSPRSMDCWGQGTSVSVSS

SEQ ID NO: 8 - protein, 109 aa, synthetic construct
  REGION 1..109: note = L Chain V Region of 1A1-2 antibody
SIVMTQTPKFLLVSAGDRVTITCKASQSVTNDVAWYQQKPGQSPKLLIYYASNRYTGVPDRFTGSGYGTDFTFTISTVQAEDLAVYFCQQDYSSPYTFGGGTMLEIKRA

SEQ ID NO: 9 - protein, 459 aa, synthetic construct
  REGION 1..459: note = H Chain V Region of 1A1-2 antibody / cat H Chain constant region
QIQLVQSGPELKKPGETVKISCKASGYTFTDYSIHWVKQAPGKGLKWMGWINTETGEPTYADDFKGRFAFSLETSVSAAFLQINNLKNEDTATYFCARPLFYYYITSPRSMDCWGQGTSVSVSSASTTAPSVFPLAPSCGTTSGATVALACLVLGYFPEPVTVSWNSGALTSGVHTFPSVLQASGLYSLSSMVTVPSSRWLSDTFTCNVAHPPSNTKVDKTVRKTDHPPGPKPCDCPKCPPPEMLGGPSIFIFPPKPKDTLSISRTPEVTCLVVDLGPDDSDVQITWFVDNTQVYTAKTSPREEQFNSTYRVVSVLPILHQDWLKGKEFKCKVNSKSLPSPIERTISKAKGQPHEPQVYVLPPAQEELSRNKVSVTCLIKSFHPPDIAVEWEITGQPEPENNYRTTPPQLDSDGTYFVYSKLSVDRSHWQRGNTYTCSVSHEALHSHHTQKSLTQSPGK

SEQ ID NO: 10 - protein, 217 aa, synthetic construct
  REGION 1..217: note = L Chain of 1A1-2 antibody / cat L Chain constant region
SIVMTQTPKFLLVSAGDRVTITCKASQSVTNDVAWYQQKPGQSPKLLIYYASNRYTGVPDRFTGSGYGTDFTFTISTVQAEDLAVYFCQQDYSSPYTFGGGTMLEIKRSDAQPSVFLFQPSLDELHTGSASIVCILNDFYPKEVNVKWKVDGVVQNKGIQESTTEQNSKDSTYSLSSTLTMSSTEYQSHEKFSCEVTHKSLASTLVKSFNRSECQRE

SEQ ID NO: 11 - protein, 278 aa, Felis silvestris
MGTPRAPWPLVWAVLQLGWWPGWLLDSPYRPWSPLTFSPAQLTVLEGENATFVCHLPDVPESFVLNWYRVSPRNQTDKLAAFQENHTEPGKDRRFRVTRLPSGQDFHTTILAAQLNDSGIYLCGAIYLPPNTQIYESPRAELTVKERVLEPPTESPSPPPRLTGQGQGLVVGVTSVLVGVLLLLLLTWVLAAAFPRATRGACACGSEDEPLKEGPSAAPVFTVDYGELDFQWREKTPEPPAPCAPEQTEYATIVFPSRPGSPGPLPLRPEDGPCPWPL

SEQ ID NO: 12 - DNA, 837 bp, Felis silvestris
  source 1..837: mol_type = other DNA
atggggaccccacgggcgccctggcctcttgtctgggccgtgctgcagctgggctggtggccaggatggctcttagactccccctacaggccctggagccccctcaccttctccccggcccagctcacggtgctcgagggggagaacgccaccttcgtctgccacctgcccgacgtacccgagagcttcgtgctcaactggtaccgcgtgagtccccgcaaccagacggacaagctggccgccttccaggagaaccacaccgagcccggcaaggacaggcgcttccgcgtcacgcggctgcccagcgggcaggacttccacacgaccatcctcgccgcccagctcaacgacagcggcatctacctctgcggggccatctacctgccccccaacacgcagatctatgagagcccacgagcggagctcactgtgaaagagagagtcctggagccccccacagagagtcccagccccccacccagactcaccggccaaggccaggggctggtcgtgggcgtcacaagcgtgctggtgggtgtcctgctgttgctgctgctgacctgggtgctggctgcggccttccccagggccactcgaggtgcctgtgcctgcgggagcgaggacgagcctctgaaggagggcccctctgcggcacccgtgttcaccgtggactacggagagctggactttcagtggcgagagaagacgcccgagccccccgccccctgcgcccccgaacagaccgagtatgccacgatcgtcttccccagcaggccgggctccccggggcccctgcctctgaggcccgaggacggaccctgcccttggcccctctga

SEQ ID NO: 13 - DNA, 28 bp, synthetic construct
  misc_feature 1..28: note = Forward primer 1
  source 1..28: mol_type = other DNA
gtggatcccgtggaggaagagattacgg

SEQ ID NO: 14 - DNA, 27 bp, synthetic construct
  misc_feature 1..27: note = Reverse primer 1
  source 1..27: mol_type = other DNA
tcgaattccgagaggagagccaagctg

SEQ ID NO: 15 - DNA, 21 bp, synthetic construct
  misc_feature 1..21: note = Forward primer 2
  source 1..21: mol_type = other DNA
ccaccgccctcaaagtagacg

SEQ ID NO: 16 - DNA, 20 bp, synthetic construct
  misc_feature 1..20: note = Reverse primer 2
  source 1..20: mol_type = other DNA
cctcacattgccaaaagacg

SEQ ID NO: 17 - DNA, 39 bp, synthetic construct
  misc_feature 1..39: note = Reverse primer 3
  source 1..39: mol_type = other DNA
gtcgatgtcatgatctttataatcgaggggccaagggca

SEQ ID NO: 18 - DNA, 36 bp, synthetic construct
  misc_feature 1..36: note = Reverse primer 4
  source 1..36: mol_type = other DNA
gtcgatgtcatgatctttataatcgtcgatgtcatg

SEQ ID NO: 19 - DNA, 28 bp, synthetic construct
  misc_feature 1..28: note = Forward primer 3
  source 1..28: mol_type = other DNA
tcgaattccagctcattagcgcgagaac

SEQ ID NO: 20 - DNA, 32 bp, synthetic construct
  misc_feature 1..32: note = Reverse primer 5
  source 1..32: mol_type = other DNA
ccctcgagttacgtctcctcaaattgtagatc

SEQ ID NO: 21 - DNA, 19 bp, synthetic construct
  misc_feature 1..19: note = Forward primer 4
  source 1..19: mol_type = other DNA
gtttacgatcacagtgtcc

SEQ ID NO: 22 - DNA, 39 bp, synthetic construct
  misc_feature 1..39: note = Reverse primer 6
  source 1..39: mol_type = other DNA
gtcgatgtcatgatctttataatccgtctcctcaaattg

SEQ ID NO: 23 - DNA, 26 bp, synthetic construct
  misc_feature 1..26: note = Reverse primer 7
  source 1..26: mol_type = other DNA
cgagatctagtcctctcatttgctgg